European Patent Application EP 4 725 956 A1, published April 15, 2026. Title: 经修饰的多肽及其在镇痛领域的应用. Applicant: 南京安吉生物科技有限公司. The sequence listing filed with the application follows.

SEQUENCE LISTING (34 sequences)

SEQ ID NO: 1 - protein, 13 aa, synthetic construct
  DISULFID 3..9: note = interchain disulfide bond
  SITE 9: note = D-Cysteine
GSCSTPPSXVLYS

SEQ ID NO: 2 - protein, 13 aa, synthetic construct
  SITE 5: note = D-Threonine
  SITE 9: note = D-cysteine
  DISULFID 3..9: note = interchain disulfide bond
GSCSXPPSXVLYS

SEQ ID NO: 3 - protein, 13 aa, synthetic construct
  DISULFID 3..9: note = interchain disulfide bond
  SITE 5: note = D-Threonine
  SITE 9: note = D-Cysteine
  SITE 13: note = Serine-NH2
GSCSXPPSXVLYX

SEQ ID NO: 4 - protein, 13 aa, synthetic construct
  DISULFID 3..9: note = interchain disulfide bond
  SITE 3: note = D-Cysteine
  SITE 5: note = D-Threonine
  SITE 9: note = D-Cysteine
GSXSXPPSXVLYS

SEQ ID NO: 5 - skipped

SEQ ID NO: 6 - protein, 13 aa, synthetic construct
  DISULFID 3..9: note = interchain disulfide bond
  SITE 1: note = Sarcosine
  SITE 5: note = D-threonine
  SITE 9: note = D-cysteine
XSCSXPPSXVLYS

SEQ ID NO: 7 - protein, 13 aa, synthetic construct
  DISULFID 3..9: note = interchain disulfide bond
  SITE 5: note = D-threonine
  SITE 9: note = D-cysteine
ASCSXPPSXVLYS

SEQ ID NO: 8 - protein, 13 aa, synthetic construct
  DISULFID 3..9: note = interchain disulfide bond
  SITE 5: note = D-threonine
  SITE 9: note = D-cysteine
GACSXPPSXVLYS

SEQ ID NO: 9 - protein, 13 aa, synthetic construct
  DISULFID 3..9: note = interchain disulfide bond
  SITE 5: note = D-threonine
  SITE 9: note = D-cysteine
GSCAXPPSXVLYS

SEQ ID NO: 10 - protein, 13 aa, synthetic construct
  DISULFID 3..9: note = interchain disulfide bond
  SITE 5: note = D-threonine
  SITE 6: note = Hydroxyproline
  SITE 9: note = D-cysteine
GSCSXXPSXVLYS

SEQ ID NO: 11 - protein, 13 aa, synthetic construct
  DISULFID 3..9: note = interchain disulfide bond
  SITE 5: note = D-threonine
  SITE 7: note = Hydroxyproline
  SITE 9: note = D-cysteine
GSCSXPXSXVLYS

SEQ ID NO: 12 - protein, 13 aa, synthetic construct
  DISULFID 3..9: note = interchain disulfide bond
  SITE 5: note = D-threonine
  SITE 9: note = D-cysteine
GSCSXPPAXVLYS

SEQ ID NO: 13 - protein, 13 aa, synthetic construct
  DISULFID 3..9: note = interchian disulfide bond
  SITE 5: note = D-threonine
  SITE 9: note = D-cysteine
GSCSXPPSXALYS

SEQ ID NO: 14 - protein, 13 aa, synthetic construct
  DISULFID 3..9: note = interchain disulfide bond
  SITE 5: note = D-threonine
  SITE 9: note = D-cysteine
GSCSXPPSXVAYS

SEQ ID NO: 15 - protein, 13 aa, synthetic construct
  DISULFID 3..9: note = interchain disulfide bond
  SITE 5: note = D-threonine
  SITE 9: note = D-cystenine
GSCSXPPSXVLAS

SEQ ID NO: 16 - protein, 13 aa, synthetic construct
  DISULFID 3..9: note = interchain disulfide bond
  SITE 5: note = D-threonine
  SITE 9: note = D-cystenine
GSCSXPPSXVLYA

SEQ ID NO: 17 - protein, 13 aa, synthetic construct
  DISULFID 3..9: note = interchain disulfide bond
  SITE 5: note = D-threonine
  SITE 9: note = D-cystenine
GSCSXPPGXVLYS

SEQ ID NO: 18 - protein, 13 aa, synthetic construct
  DISULFID 3..9: note = interchain disulfide bond
  SITE 5: note = D-threonine
  SITE 9: note = D-cystenine
  SITE 10: note = Aib
GSCSXPPSXXLYS

SEQ ID NO: 19 - protein, 13 aa, synthetic construct
  DISULFID 3..9: note = interchain disulfide bond
  SITE 5: note = D-threonine
  SITE 9: note = D-cystenine
GSCSXPPSXGLYS

SEQ ID NO: 20 - protein, 13 aa, synthetic construct
  SITE 5: note = D-threonine
  SITE 9: note = D-cystenine
  DISULFID 3..9: note = interchain disulfide bond
GSCSXPPSXVIYS

SEQ ID NO: 21 - protein, 13 aa, synthetic construct
  DISULFID 3..9: note = interchain disulfide bond
  SITE 5: note = D-threonine
  SITE 9: note = D-cystenine
  SITE 11: note = ABu
GSCSXPPSXVXYS

SEQ ID NO: 22 - protein, 13 aa, synthetic construct
  DISULFID 3..9: note = interchain disulfide bond
  SITE 5: note = D-threonine
  SITE 9: note = D-cystenine
  SITE 11: note = Nle
GSCSXPPSXVXYS

SEQ ID NO: 23 - protein, 13 aa, synthetic construct
  DISULFID 3..9: note = interchain disulfide bond
  SITE 5: note = D-threonine
  SITE 9: note = D-cystenine
GSCSXPPSXVLWS

SEQ ID NO: 24 - protein, 13 aa, synthetic construct
  DISULFID 3..9: note = interchain disulfide bond
  SITE 5: note = D-threonine
  SITE 9: note = D-cystenine
  SITE 12: note = Biphenylalanine
GSCSXPPSXVLXS

SEQ ID NO: 25 - protein, 13 aa, synthetic construct
  DISULFID 3..9: note = interchain disulfide bond
  SITE 5: note = D-threonine
  SITE 9: note = D-cystenine
  SITE 13: note = Orn-NH2
GSCSXPPSXVLYX

SEQ ID NO: 26 - protein, 13 aa, synthetic construct
  DISULFID 3..9: note = interchain disulfide bond
  SITE 5: note = D-threonine
  SITE 9: note = D-cystenine
  SITE 6: note = Hydroxyproline
  SITE 7: note = Hydroxyproline
  SITE 11: note = Nle
  SITE 12: note = Biphenylalanine
  SITE 13: note = Orn-NH2
GSCSXXXSXVXXX

SEQ ID NO: 27 - protein, 13 aa, synthetic construct
  DISULFID 3..9: note = interchain disulfide bond
  SITE 5: note = D-threonine
  SITE 6: note = Hydroxyproline
  SITE 7: note = Hydroxyproline
  SITE 9: note = D-cystenine
  SITE 11: note = Nle
  SITE 12: note = Biphenylalanine
  SITE 13: note = Orn-NH2
GSCSXXXAXVXXX

SEQ ID NO: 28 - protein, 13 aa, synthetic construct
  DISULFID 3..9: note = interchain disulfide bond
  SITE 5: note = D-threonine
  SITE 6: note = Hydroxyproline
  SITE 7: note = Hydroxyproline
  SITE 9: note = D-cystenine
  SITE 8: note = Aib
  SITE 11: note = Nle
  SITE 12: note = Biphenylalanine
  SITE 13: note = Orn-NH2
GSCSXXXXXVXXX

SEQ ID NO: 29 - protein, 13 aa, synthetic construct
  DISULFID 3..9: note = interchain disulfide bond
  SITE 5: note = D-threonine
  SITE 6: note = Hydroxyproline
  SITE 7: note = Hydroxyproline
  SITE 9: note = D-cystenine
  SITE 11: note = Nle
  SITE 13: note = Orn-NH2
GSCSXXXSXVXFX

SEQ ID NO: 30 - protein, 13 aa, synthetic construct
  DISULFID 3..9: note = interchain disulfide bond
  SITE 5: note = D-threonine
  SITE 6: note = Hydroxyproline
  SITE 7: note = Hydroxyproline
  SITE 9: note = D-cystenine
  SITE 11: note = Nle
  SITE 13: note = Orn-NH2
GSCSXXXAXVXFX

SEQ ID NO: 31 - protein, 13 aa, synthetic construct
  DISULFID 3..9: note = interchain disulfide bond
  SITE 5: note = D-threonine
  SITE 6: note = Hydroxyproline
  SITE 7: note = Hydroxyproline
  SITE 8: note = Aib
  SITE 9: note = D-cystenine
  SITE 11: note = Nle
  SITE 13: note = Orn-NH2
GSCSXXXXXVXFX

SEQ ID NO: 32 - protein, 13 aa, synthetic construct
  DISULFID 3..9: note = interchain disulfide bond
  SITE 5: note = D-threonine
  SITE 6: note = Hydroxyproline
  SITE 7: note = Hydroxyproline
  SITE 9: note = D-cystenine
  SITE 11: note = Nle
  SITE 13: note = Orn-NH2
GSCSXXXSXVXWX

SEQ ID NO: 33 - protein, 13 aa, synthetic construct
  DISULFID 3..9: note = interchain disulfide bond
  SITE 5: note = D-threonine
  SITE 6: note = Hydroxyproline
  SITE 7: note = Hydroxyproline
  SITE 9: note = D-cystenine
  SITE 11: note = Nle
  SITE 13: note = Orn-NH2
GSCSXXXAXVXWX

SEQ ID NO: 34 - protein, 13 aa, synthetic construct
  DISULFID 3..9: note = interchain disulfide bond
  SITE 5: note = D-threonine
  SITE 6: note = Hydroxyproline
  SITE 7: note = hydroxyproline
  SITE 8: note = Aib
  SITE 9: note = D-cystenine
  SITE 11: note = Nle
  SITE 13: note = Orn-NH2
GSCSXXXXXVXWX